European Patent Application EP 4 778 541 A1, published July 22, 2026. Title: 基因递送系统及其在制备肿瘤治疗药物中的应用. Applicant: 上海赛迪夫医药科技有限公司. Application CN. The sequence listing filed with the application follows.

SEQUENCE LISTING (3 sequences)

SEQ ID NO: 1 - DNA, 1425 bp, synthetic construct
  source 1..1425: mol_type = other DNA
atgcgactctccaaaaccctcgtcgacatggacatggccgactacagtgctgcactggacccagcctacaccaccctggaatttgagaatgtgcaggtgttgacgatgggcaatgacacgtccccatcagaaggcaccaacctcaacgcgcccaacagcctgggtgtcagcgccctgtgtgccatctgcggggaccgggccacgggcaaacactacggtgcctcgagctgtgacggctgcaagggcttcttccggaggagcgtgcggaagaaccacatgtactcctgcagatttagccggcagtgcgtggtggacaaagacaagaggaaccagtgccgctactgcaggctcaagaaatgcttccgggctggcatgaagaaggaagccgtccagaatgagcgggaccggatcagcactcgaaggtcaagctatgaggacagcagcctgccctccatcaatgcgctcctgcaggcggaggtcctgtcccgacagatcacctcccccgtctccgggatcaacggcgacattcgggcgaagaagattgccagcatcgcagatgtgtgtgagtccatgaaggagcagctgctggttctcgttgagtgggccaagtacatcccagctttctgcgagctccccctggacgaccaggtggccctgctcagagcccatgctggcgagcacctgctgctcggagccaccaagagatccatggtgttcaaggacgtgctgctcctaggcaatgactacattgtccctcggcactgcccggagctggcggagatgagccgggtgtccatacgcatccttgacgagctggtgctgcccttccaggagctgcagatcgatgacaatgagtatgcctacctcaaagccatcatcttctttgacccagatgccaaggggctgagcgatccagggaagatcaagcggctgcgttcccaggtgcaggtgagcttggaggactacatcaacgaccgccagtatgactcgcgtggccgctttggagagctgctgctgctgctgcccaccttgcagagcatcacctggcagatgatcgagcagatccagttcatcaagctcttcggcatggccaagattgacaacctgttgcaggagatgctgctgggagggtcccccagcgatgcaccccatgcccaccaccccctgcaccctcacctgatgcaggaacatatgggaaccaacgtcatcgttgccaacacaatgcccactcacctcagcaacggacagatgtgtgagtggccccgacccaggggacaggcagccacccctgagaccccacagccctcaccgccaggtggctcagggtctgagccctataagctcctgccgggagccgtcgccacaatcgtcaagcccctctctgccatcccccagccgaccatcaccaagcaggaagttatctag

SEQ ID NO: 2 - DNA, 7695 bp, synthetic construct
  source 1..7695: mol_type = other DNA
ataggcggcgcatgagagaagcccagaccaattacctacccaaaatggagaaagttcacgttgacatcgaggaagacagcccattcctcagagctttgcagcggagcttcccgcagtttgaggtagaagccaagcaggtcactgataatgaccatgctaatgccagagcgttttcgcatctggcttcaaaactgatcgaaacggaggtggacccatccgacacgatccttgacattggaagtgcgcccgcccgcagaatgtattctaagcacaagtatcattgtatctgtccgatgagatgtgcggaagatccggacagattgtataagtatgcaactaagctgaagaaaaactgtaaggaaataactgataaggaattggacaagaaaatgaaggagctcgccgccgtcatgagcgaccctgacctggaaactgagactatgtgcctccacgacgacgagtcgtgtcgctacgaagggcaagtcgctgtttaccaggatgtatacgcggttgacggaccgacaagtctctatcaccaagccaataagggagttagagtcgcctactggataggctttgacaccaccccttttatgtttaagaacttggctggagcatatccatcatactctaccaactgggccgacgaaaccgtgttaacggctcgtaacataggcctatgcagctctgacgttatggagcggtcacgtagagggatgtccattcttagaaagaagtatttgaaaccatccaacaatgttctattctctgttggctcgaccatctaccacgagaagagggacttactgaggagctggcacctgccgtctgtatttcacttacgtggcaagcaaaattacacatgtcggtgtgagactatagttagttgcgacgggtacgtcgttaaaagaatagctatcagtccaggcctgtatgggaagccttcaggctatgctgctacgatgcaccgcgagggattcttgtgctgcaaagtgacagacacattgaacggggagagggtctcttttcccgtgtgcacgtatgtgccagctacattgtgtgaccaaatgactggcatactggcaacagatgtcagtgcggacgacgcgcaaaaactgctggttgggctcaaccagcgtatagtcgtcaacggtcgcacccagagaaacaccaataccatgaaaaattaccttttgcccgtagtggcccaggcatttgctaggtgggcaaaggaatataaggaagatcaagaagatgaaaggccactaggactacgagatagacagttagtcatggggtgttgttgggcttttagaaggcacaagataacatctatttataagcgcccggatacccaaaccatcatcaaagtgaacagcgatttccactcattcgtgctgcccaggataggcagtaacacattggagatcgggctgagaacaagaatcaggaaaatgttagaggagcacaaggagccgtcacctctcattaccgccgaggacgtacaagaagctaagtgcgcagccgatgaggctaaggaggtgcgtgaagccgaggagttgcgcgcagctctaccacctttggcagctgatgttgaggagcccactctggaagccgatgtcgacttgatgttacaagaggctggggccggctcagtggagacacctcgtggcttgataaaggttaccagctacgatggcgaggacaagatcggctcttacgctgtgctttctccgcaggctgtactcaagagtgaaaaattatcttgcatccaccctctcgctgaacaagtcatagtgataacacactctggccgaaaagggcgttatgccgtggaaccataccatggtaaagtagtggtgccagagggacatgcaatacccgtccaggactttcaagctctgagtgaaagtgccaccattgtgtacaacgaacgtgagttcgtaaacaggtacctgcaccatattgccacacatggaggagcgctgaacactgatgaagaatattacaaaactgtcaagcccagcgagcacgacggcgaatacctgtacgacatcgacaggaaacagtgcgtcaagaaagaactagtcactgggctagggctcacaggcgagctggtggatcctcccttccatgaattcgcctacgagagtctgagaacacgaccagccgctccttaccaagtaccaaccataggggtgtatggcgtgccaggatcaggcaagtctggcatcattaaaagcgcagtcaccaaaaaagatctagtggtgagcgccaagaaagaaaactgtgcagaaattataagggacgtcaagaaaatgaaagggctggacgtcaatgccagaactgtggactcagtgctcttgaatggatgcaaacaccccgtagagaccctgtatattgacgaagcttttgcttgtcatgcaggtactctcagagcgctcatagccattataagacctaaaaaggcagtgctctgcggggatcccaaacagtgcggtttttttaacatgatgtgcctgaaagtgcattttaaccacgagatttgcacacaagtcttccacaaaagcatctctcgccgttgcactaaatctgtgacttcggtcgtctcaaccttgttttacgacaaaaaaatgagaacgacgaatccgaaagagactaagattgtgattgacactaccggcagtaccaaacctaagcaggacgatctcattctcacttgtttcagagggtgggtgaagcagttgcaaatagattacaaaggcaacgaaataatgacggcagctgcctctcaagggctgacccgtaaaggtgtgtatgccgttcggtacaaggtgaatgaaaatcctctgtacgcacccacctcagaacatgtgaacgtcctactgacccgcacggaggaccgcatcgtgtggaaaacactagccggcgacccatggataaaaacactgactgccaagtaccctgggaatttcactgccacgatagaggagtggcaagcagagcatgatgccatcatgaggcacatcttggagagaccggaccctaccgacgtcttccagaataaggcaaacgtgtgttgggccaaggctttagtgccggtgctgaagaccgctggcatagacatgaccactgaacaatggaacactgtggattattttgaaacggacaaagctcactcagcagagatagtattgaaccaactatgcgtgaggttctttggactcgatctggactccggtctattttctgcacccactgttccgttatccattaggaataatcactgggataactccccgtcgcctaacatgtacgggctgaataaagaagtggtccgtcagctctctcgcaggtacccacaactgcctcgggcagttgccactggaagagtctatgacatgaacactggtacactgcgcaattatgatccgcgcataaacctagtacctgtaaacagaagactgcctcatgctttagtcctccaccataatgaacacccacagagtgacttttcttcattcgtcagcaaattgaagggcagaactgtcctggtggtcggggaaaagttgtccgtcccaggcaaaatggttgactggttgtcagaccggcctgaggctaccttcagagctcggctggatttaggcatcccaggtgatgtgcccaaatatgacataatatttgttaatgtgaggaccccatataaataccatcactatcagcagtgtgaagaccatgccattaagcttagcatgttgaccaagaaagcttgtctgcatctgaatcccggcggaacctgtgtcagcataggttatggttacgctgacagggccagcgaaagcatcattggtgctatagcgcggcagttcaagttttcccgggtatgcaaaccgaaatcctcacttgaagagacggaagttctgtttgtattcattgggtacgatcgcaaggcccgtacgcacaatccttacaagctttcatcaaccttgaccaacatttatacaggttccagactccacgaagccggatgtgcaccctcatatcatgtggtgcgaggggatattgccacggccaccgaaggagtgattataaatgctgctaacagcaaaggacaacctggcggaggggtgtgcggagcgctgtataagaaattcccggaaagcttcgatttacagccgatcgaagtaggaaaagcgcgactggtcaaaggtgcagctaaacatatcattcatgccgtaggaccaaacttcaacaaagtttcggaggttgaaggtgacaaacagttggcagaggcttatgagtccatcgctaagattgtcaacgataacaattacaagtcagtagcgattccactgttgtccaccggcatcttttccgggaacaaagatcgactaacccaatcattgaaccatttgctgacagctttagacaccactgatgcagatgtagccatatactgcagggacaagaaatgggaaatgactctcaaggaagcagtggctaggagagaagcagtggaggagatatgcatatccgacgactcttcagtgacagaacctgatgcagagctggtgagggtgcatccgaagagttctttggctggaaggaagggctacagcacaagcgatggcaaaactttctcatatttggaagggaccaagtttcaccaggcggccaaggatatagcagaaattaatgccatgtggcccgttgcaacggaggccaatgagcaggtatgcatgtatatcctcggagaaagcatgagcagtattaggtcgaaatgccccgtcgaagagtcggaagcctccacaccacctagcacgctgccttgcttgtgcatccatgccatgactccagaaagagtacagcgcctaaaagcctcacgtccagaacaaattactgtgtgctcatcctttccattgccgaagtatagaatcactggtgtgcagaagatccaatgctcccagcctatattgttctcaccgaaagtgcctgcgtatattcatccaaggaagtatctcgtggaaacaccaccggtagacgagactccggagccatcggcagagaaccaatccacagaggggacacctgaacaaccaccacttataaccgaggatgagaccaggactagaacgcctgagccgatcatcatcgaagaggaagaagaggatagcataagtttgctgtcagatggcccgacccaccaggtgctgcaagtcgaggcagacattcacgggccgccctctgtatctagctcatcctggtccattcctcatgcatccgactttgatgtggacagtttatccatacttgacaccctggagggagctagcgtgaccagcggggcaacgtcagccgagactaactcttacttcgcaaagagtatggagtttctggcgcgaccggtgcctgcgcctcgaacagtattcaggaaccctccacatcccgctccgcgcacaagaacaccgtcacttgcacccagcagggcctgctcgagaaccagcctagtttccaccccgccaggcgtgaatagggtgatcactagagaggagctcgaggcgcttaccccgtcacgcactcctagcaggtcggtctcgagaaccagcctggtctccaacccgccaggcgtaaatagggtgattacaagagaggagtttgaggcgttcgtagcacaacaacaatgacggtttgatgcgggtgcatacatcttttcctccgacaccggtcaagggcatttacaacaaaaatcagtaaggcaaacggtgctatccgaagtggtgttggagaggaccgaattggagatttcgtatgccccgcgcctcgaccaagaaaaagaagaattactacgcaagaaattacagttaaatcccacacctgctaacagaagcagataccagtccaggaaggtggagaacatgaaagccataacagctagacgtattctgcaaggcctagggcattatttgaaggcagaaggaaaagtggagtgctaccgaaccctgcatcctgttcctttgtattcatctagtgtgaaccgtgccttttcaagccccaaggtcgcagtggaagcctgtaacgccatgttgaaagagaactttccgactgtggcttcttactgtattattccagagtacgatgcctatttggacatggttgacggagcttcatgctgcttagacactgccagtttttgccctgcaaagctgcgcagctttccaaagaaacactcctatttggaacccacaatacgatcggcagtgccttcagcgatccagaacacgctccagaacgtcctggcagctgccacaaaaagaaattgcaatgtcacgcaaatgagagaattgcccgtattggattcggcggcctttaatgtggaatgcttcaagaaatatgcgtgtaataatgaatattgggaaacgtttaaagaaaaccccatcaggcttactgaagaaaacgtggtaaattacattaccaaattaaaaggaccaaaagctgctgctctttttgcgaagacacataatttgaatatgttgcaggacataccaatggacaggtttgtaatggacttaaagagagacgtgaaagtgactccaggaacaaaacatactgaagaacggcccaaggtacaggtgatccaggctgccgatccgctagcaacagcgtatctgtgcggaatccaccgagagctggttaggagattaaatgcggtcctgcttccgaacattcatacactgtttgatatgtcggctgaagactttgacgctattatagccgagcacttccagcctggggattgtgttctggaaactgacatcgcgtcgtttgataaaagtgaggacgacgccatggctctgaccgcgttaatgattctggaagacttaggtgtggacgcagagctgttgacgctgattgaggcggctttcggcgaaatttcatcaatacatttgcccactaaaactaaatttaaattcggagccatgatgaaatctggaatgttcctcacactgtttgtgaacacagtcattaacattgtaatcgcaagcagagtgttgagagaacggctaaccggatcaccatgtgcagcattcattggagatgacaatatcgtgaaaggagtcaaatcggacaaattaatggcagacaggtgcgccacctggttgaatatggaagtcaagattatagatgctgtggtgggcgagaaagcgccttatttctgtggagggtttattttgtgtgactccgtgaccggcacagcgtgccgtgtggcagaccccctaaaaaggctgtttaagcttggcaaacctctggcagcagacgatgaacatgatgatgacaggagaagggcattgcatgaagagtcaacacgctggaaccgagtgggtattctttcagagctgtgcaaggcagtagaatcaaggtatgaaaccgtaggaacttccatcatagttatggccatgactactctagctagcagtgttaaatcattcagctacctgagaggggccggccgcatacagcagcaattggcaagctgcttacatagaactcgcggcgattggcatgccgccttaaaatttttattttatttttcttttcttttccgaatcggattttgtttttaatatttcaaaaaaaaaaaaaaaaaaaaaaaaaaaaaaaaaaaaaaaaaaaaaaaaaaaaaaaaaaaaaaaaaaa

SEQ ID NO: 3 - DNA, 9120 bp, synthetic construct
  source 1..9120: mol_type = other DNA
ataggcggcgcatgagagaagcccagaccaattacctacccaaaatggagaaagttcacgttgacatcgaggaagacagcccattcctcagagctttgcagcggagcttcccgcagtttgaggtagaagccaagcaggtcactgataatgaccatgctaatgccagagcgttttcgcatctggcttcaaaactgatcgaaacggaggtggacccatccgacacgatccttgacattggaagtgcgcccgcccgcagaatgtattctaagcacaagtatcattgtatctgtccgatgagatgtgcggaagatccggacagattgtataagtatgcaactaagctgaagaaaaactgtaaggaaataactgataaggaattggacaagaaaatgaaggagctcgccgccgtcatgagcgaccctgacctggaaactgagactatgtgcctccacgacgacgagtcgtgtcgctacgaagggcaagtcgctgtttaccaggatgtatacgcggttgacggaccgacaagtctctatcaccaagccaataagggagttagagtcgcctactggataggctttgacaccaccccttttatgtttaagaacttggctggagcatatccatcatactctaccaactgggccgacgaaaccgtgttaacggctcgtaacataggcctatgcagctctgacgttatggagcggtcacgtagagggatgtccattcttagaaagaagtatttgaaaccatccaacaatgttctattctctgttggctcgaccatctaccacgagaagagggacttactgaggagctggcacctgccgtctgtatttcacttacgtggcaagcaaaattacacatgtcggtgtgagactatagttagttgcgacgggtacgtcgttaaaagaatagctatcagtccaggcctgtatgggaagccttcaggctatgctgctacgatgcaccgcgagggattcttgtgctgcaaagtgacagacacattgaacggggagagggtctcttttcccgtgtgcacgtatgtgccagctacattgtgtgaccaaatgactggcatactggcaacagatgtcagtgcggacgacgcgcaaaaactgctggttgggctcaaccagcgtatagtcgtcaacggtcgcacccagagaaacaccaataccatgaaaaattaccttttgcccgtagtggcccaggcatttgctaggtgggcaaaggaatataaggaagatcaagaagatgaaaggccactaggactacgagatagacagttagtcatggggtgttgttgggcttttagaaggcacaagataacatctatttataagcgcccggatacccaaaccatcatcaaagtgaacagcgatttccactcattcgtgctgcccaggataggcagtaacacattggagatcgggctgagaacaagaatcaggaaaatgttagaggagcacaaggagccgtcacctctcattaccgccgaggacgtacaagaagctaagtgcgcagccgatgaggctaaggaggtgcgtgaagccgaggagttgcgcgcagctctaccacctttggcagctgatgttgaggagcccactctggaagccgatgtcgacttgatgttacaagaggctggggccggctcagtggagacacctcgtggcttgataaaggttaccagctacgatggcgaggacaagatcggctcttacgctgtgctttctccgcaggctgtactcaagagtgaaaaattatcttgcatccaccctctcgctgaacaagtcatagtgataacacactctggccgaaaagggcgttatgccgtggaaccataccatggtaaagtagtggtgccagagggacatgcaatacccgtccaggactttcaagctctgagtgaaagtgccaccattgtgtacaacgaacgtgagttcgtaaacaggtacctgcaccatattgccacacatggaggagcgctgaacactgatgaagaatattacaaaactgtcaagcccagcgagcacgacggcgaatacctgtacgacatcgacaggaaacagtgcgtcaagaaagaactagtcactgggctagggctcacaggcgagctggtggatcctcccttccatgaattcgcctacgagagtctgagaacacgaccagccgctccttaccaagtaccaaccataggggtgtatggcgtgccaggatcaggcaagtctggcatcattaaaagcgcagtcaccaaaaaagatctagtggtgagcgccaagaaagaaaactgtgcagaaattataagggacgtcaagaaaatgaaagggctggacgtcaatgccagaactgtggactcagtgctcttgaatggatgcaaacaccccgtagagaccctgtatattgacgaagcttttgcttgtcatgcaggtactctcagagcgctcatagccattataagacctaaaaaggcagtgctctgcggggatcccaaacagtgcggtttttttaacatgatgtgcctgaaagtgcattttaaccacgagatttgcacacaagtcttccacaaaagcatctctcgccgttgcactaaatctgtgacttcggtcgtctcaaccttgttttacgacaaaaaaatgagaacgacgaatccgaaagagactaagattgtgattgacactaccggcagtaccaaacctaagcaggacgatctcattctcacttgtttcagagggtgggtgaagcagttgcaaatagattacaaaggcaacgaaataatgacggcagctgcctctcaagggctgacccgtaaaggtgtgtatgccgttcggtacaaggtgaatgaaaatcctctgtacgcacccacctcagaacatgtgaacgtcctactgacccgcacggaggaccgcatcgtgtggaaaacactagccggcgacccatggataaaaacactgactgccaagtaccctgggaatttcactgccacgatagaggagtggcaagcagagcatgatgccatcatgaggcacatcttggagagaccggaccctaccgacgtcttccagaataaggcaaacgtgtgttgggccaaggctttagtgccggtgctgaagaccgctggcatagacatgaccactgaacaatggaacactgtggattattttgaaacggacaaagctcactcagcagagatagtattgaaccaactatgcgtgaggttctttggactcgatctggactccggtctattttctgcacccactgttccgttatccattaggaataatcactgggataactccccgtcgcctaacatgtacgggctgaataaagaagtggtccgtcagctctctcgcaggtacccacaactgcctcgggcagttgccactggaagagtctatgacatgaacactggtacactgcgcaattatgatccgcgcataaacctagtacctgtaaacagaagactgcctcatgctttagtcctccaccataatgaacacccacagagtgacttttcttcattcgtcagcaaattgaagggcagaactgtcctggtggtcggggaaaagttgtccgtcccaggcaaaatggttgactggttgtcagaccggcctgaggctaccttcagagctcggctggatttaggcatcccaggtgatgtgcccaaatatgacataatatttgttaatgtgaggaccccatataaataccatcactatcagcagtgtgaagaccatgccattaagcttagcatgttgaccaagaaagcttgtctgcatctgaatcccggcggaacctgtgtcagcataggttatggttacgctgacagggccagcgaaagcatcattggtgctatagcgcggcagttcaagttttcccgggtatgcaaaccgaaatcctcacttgaagagacggaagttctgtttgtattcattgggtacgatcgcaaggcccgtacgcacaatccttacaagctttcatcaaccttgaccaacatttatacaggttccagactccacgaagccggatgtgcaccctcatatcatgtggtgcgaggggatattgccacggccaccgaaggagtgattataaatgctgctaacagcaaaggacaacctggcggaggggtgtgcggagcgctgtataagaaattcccggaaagcttcgatttacagccgatcgaagtaggaaaagcgcgactggtcaaaggtgcagctaaacatatcattcatgccgtaggaccaaacttcaacaaagtttcggaggttgaaggtgacaaacagttggcagaggcttatgagtccatcgctaagattgtcaacgataacaattacaagtcagtagcgattccactgttgtccaccggcatcttttccgggaacaaagatcgactaacccaatcattgaaccatttgctgacagctttagacaccactgatgcagatgtagccatatactgcagggacaagaaatgggaaatgactctcaaggaagcagtggctaggagagaagcagtggaggagatatgcatatccgacgactcttcagtgacagaacctgatgcagagctggtgagggtgcatccgaagagttctttggctggaaggaagggctacagcacaagcgatggcaaaactttctcatatttggaagggaccaagtttcaccaggcggccaaggatatagcagaaattaatgccatgtggcccgttgcaacggaggccaatgagcaggtatgcatgtatatcctcggagaaagcatgagcagtattaggtcgaaatgccccgtcgaagagtcggaagcctccacaccacctagcacgctgccttgcttgtgcatccatgccatgactccagaaagagtacagcgcctaaaagcctcacgtccagaacaaattactgtgtgctcatcctttccattgccgaagtatagaatcactggtgtgcagaagatccaatgctcccagcctatattgttctcaccgaaagtgcctgcgtatattcatccaaggaagtatctcgtggaaacaccaccggtagacgagactccggagccatcggcagagaaccaatccacagaggggacacctgaacaaccaccacttataaccgaggatgagaccaggactagaacgcctgagccgatcatcatcgaagaggaagaagaggatagcataagtttgctgtcagatggcccgacccaccaggtgctgcaagtcgaggcagacattcacgggccgccctctgtatctagctcatcctggtccattcctcatgcatccgactttgatgtggacagtttatccatacttgacaccctggagggagctagcgtgaccagcggggcaacgtcagccgagactaactcttacttcgcaaagagtatggagtttctggcgcgaccggtgcctgcgcctcgaacagtattcaggaaccctccacatcccgctccgcgcacaagaacaccgtcacttgcacccagcagggcctgctcgagaaccagcctagtttccaccccgccaggcgtgaatagggtgatcactagagaggagctcgaggcgcttaccccgtcacgcactcctagcaggtcggtctcgagaaccagcctggtctccaacccgccaggcgtaaatagggtgattacaagagaggagtttgaggcgttcgtagcacaacaacaatgacggtttgatgcgggtgcatacatcttttcctccgacaccggtcaagggcatttacaacaaaaatcagtaaggcaaacggtgctatccgaagtggtgttggagaggaccgaattggagatttcgtatgccccgcgcctcgaccaagaaaaagaagaattactacgcaagaaattacagttaaatcccacacctgctaacagaagcagataccagtccaggaaggtggagaacatgaaagccataacagctagacgtattctgcaaggcctagggcattatttgaaggcagaaggaaaagtggagtgctaccgaaccctgcatcctgttcctttgtattcatctagtgtgaaccgtgccttttcaagccccaaggtcgcagtggaagcctgtaacgccatgttgaaagagaactttccgactgtggcttcttactgtattattccagagtacgatgcctatttggacatggttgacggagcttcatgctgcttagacactgccagtttttgccctgcaaagctgcgcagctttccaaagaaacactcctatttggaacccacaatacgatcggcagtgccttcagcgatccagaacacgctccagaacgtcctggcagctgccacaaaaagaaattgcaatgtcacgcaaatgagagaattgcccgtattggattcggcggcctttaatgtggaatgcttcaagaaatatgcgtgtaataatgaatattgggaaacgtttaaagaaaaccccatcaggcttactgaagaaaacgtggtaaattacattaccaaattaaaaggaccaaaagctgctgctctttttgcgaagacacataatttgaatatgttgcaggacataccaatggacaggtttgtaatggacttaaagagagacgtgaaagtgactccaggaacaaaacatactgaagaacggcccaaggtacaggtgatccaggctgccgatccgctagcaacagcgtatctgtgcggaatccaccgagagctggttaggagattaaatgcggtcctgcttccgaacattcatacactgtttgatatgtcggctgaagactttgacgctattatagccgagcacttccagcctggggattgtgttctggaaactgacatcgcgtcgtttgataaaagtgaggacgacgccatggctctgaccgcgttaatgattctggaagacttaggtgtggacgcagagctgttgacgctgattgaggcggctttcggcgaaatttcatcaatacatttgcccactaaaactaaatttaaattcggagccatgatgaaatctggaatgttcctcacactgtttgtgaacacagtcattaacattgtaatcgcaagcagagtgttgagagaacggctaaccggatcaccatgtgcagcattcattggagatgacaatatcgtgaaaggagtcaaatcggacaaattaatggcagacaggtgcgccacctggttgaatatggaagtcaagattatagatgctgtggtgggcgagaaagcgccttatttctgtggagggtttattttgtgtgactccgtgaccggcacagcgtgccgtgtggcagaccccctaaaaaggctgtttaagcttggcaaacctctggcagcagacgatgaacatgatgatgacaggagaagggcattgcatgaagagtcaacacgctggaaccgagtgggtattctttcagagctgtgcaaggcagtagaatcaaggtatgaaaccgtaggaacttccatcatagttatggccatgactactctagctagcagtgttaaatcattcagctacctgagaggggccatgcgactctccaaaaccctcgtcgacatggacatggccgactacagtgctgcactggacccagcctacaccaccctggaatttgagaatgtgcaggtgttgacgatgggcaatgacacgtccccatcagaaggcaccaacctcaacgcgcccaacagcctgggtgtcagcgccctgtgtgccatctgcggggaccgggccacgggcaaacactacggtgcctcgagctgtgacggctgcaagggcttcttccggaggagcgtgcggaagaaccacatgtactcctgcagatttagccggcagtgcgtggtggacaaagacaagaggaaccagtgccgctactgcaggctcaagaaatgcttccgggctggcatgaagaaggaagccgtccagaatgagcgggaccggatcagcactcgaaggtcaagctatgaggacagcagcctgccctccatcaatgcgctcctgcaggcggaggtcctgtcccgacagatcacctcccccgtctccgggatcaacggcgacattcgggcgaagaagattgccagcatcgcagatgtgtgtgagtccatgaaggagcagctgctggttctcgttgagtgggccaagtacatcccagctttctgcgagctccccctggacgaccaggtggccctgctcagagcccatgctggcgagcacctgctgctcggagccaccaagagatccatggtgttcaaggacgtgctgctcctaggcaatgactacattgtccctcggcactgcccggagctggcggagatgagccgggtgtccatacgcatccttgacgagctggtgctgcccttccaggagctgcagatcgatgacaatgagtatgcctacctcaaagccatcatcttctttgacccagatgccaaggggctgagcgatccagggaagatcaagcggctgcgttcccaggtgcaggtgagcttggaggactacatcaacgaccgccagtatgactcgcgtggccgctttggagagctgctgctgctgctgcccaccttgcagagcatcacctggcagatgatcgagcagatccagttcatcaagctcttcggcatggccaagattgacaacctgttgcaggagatgctgctgggagggtcccccagcgatgcaccccatgcccaccaccccctgcaccctcacctgatgcaggaacatatgggaaccaacgtcatcgttgccaacacaatgcccactcacctcagcaacggacagatgtgtgagtggccccgacccaggggacaggcagccacccctgagaccccacagccctcaccgccaggtggctcagggtctgagccctataagctcctgccgggagccgtcgccacaatcgtcaagcccctctctgccatcccccagccgaccatcaccaagcaggaagttatctagggccgcatacagcagcaattggcaagctgcttacatagaactcgcggcgattggcatgccgccttaaaatttttattttatttttcttttcttttccgaatcggattttgtttttaatatttcaaaaaaaaaaaaaaaaaaaaaaaaaaaaaaaaaaaaaaaaaaaaaaaaaaaaaaaaaaaaaaaaaaa